European Patent Application EP 4 289 861 A1, published December 13, 2023. Title: ANTIBODIES AGAINST HUMAN TSLP AND USE THEREOF. Applicant: Beijing Wisdomab Biotechnology Co., Ltd GENRIX (Shanghai) Biopharmaceutical Co., Ltd. Chongqing Genrix Biopharmaceutical Co., Ltd. Application EP21924079.3. The sequence listing filed with the application follows.

SEQUENCE LISTING (43 sequences)

SEQ ID NO: 1 - protein, 131 aa, Homo sapiens
YDFTNCDFEKIKAAYLSTISKDLITYMSGTKSTEFNNTVSCSNRPHCLTEIQSLTFNPTAGCASLAKEMFAMKTKAALAIWCPGYSETQINATQAMKKRRKRKVTTNKCLEQVSQLQGLWRRFNRPLLKQQ

SEQ ID NO: 2 - protein, 63 aa, Homo sapiens
MFAMKTKAALAIWCPGYSETQINATQAMKKRRKRKVTTNKCLEQVSQLQGLWRRFNRPLLKQQ

SEQ ID NO: 3 - protein, 121 aa, Mus musculus
YNFSNCNFTSITKIYCNIIFHDLTGDLKGAKFEQIEDCESKPACLLKIEYYTLNPIPGCPSLPDKTFARRTREALNDHCPGYPETERNDGTQEMAQEVQNICLNQTSQILRLWYSFMQSPE

SEQ ID NO: 4 - protein, 131 aa, Macaca fascicularis
YDFTNCDFQKIEADYLRTISKDLITYMSGTKSTDFNNTVSCSNRPHCLTEIQSLTFNPTPRCASLAKEMFARKTKATLALWCPGYSETQINATQAMKKRRKRKVTTNKCLEQVSQLLGLWRRFIRTLLKKQ

SEQ ID NO: 5 - protein, 126 aa, Artificial Sequence
  hTSLP1 mutant (hTSLP1-m) with the deletion of furin recognition site
YDFTNCDFEKIKAAYLSTISKDLITYMSGTKSTEFNNTVSCSNRPHCLTEIQSLTFNPTAGCASLAKEMFAMKTKAALAIWCPGYSETQINATQAMKKVTTNKCLEQVSQLQGLWRRFNRPLLKQQ

SEQ ID NO: 6 - protein, 58 aa, Artificial Sequence
  hTSLP2 mutant (hTSLP2-m) with the deletion of furin recognition site
MFAMKTKAALAIWCPGYSETQINATQAMKKVTTNKCLEQVSQLQGLWRRFNRPLLKQQ

SEQ ID NO: 7 - protein, 126 aa, Artificial Sequence
  mfTSLP mutant (mfTSLP1-m) with the deletion of furin recognition site
YDFTNCDFQKIEADYLRTISKDLITYMSGTKSTDFNNTVSCSNRPHCLTEIQSLTFNPTPRCASLAKEMFARKTKATLALWCPGYSETQINATQAMKKVTTNKCLEQVSQLLGLWRRFIRTLLKKQ

SEQ ID NO: 8 - protein, 6 aa, Artificial Sequence
  His tag
HHHHHH

SEQ ID NO: 9 - protein, 232 aa, Homo sapiens
EPKSSDKTHTCPPCPAPELLGGPSVFLFPPKPKDTLMISRTPEVTCVVVDVSHEDPEVKFNWYVDGVEVHNAKTKPREEQYNSTYRVVSVLTVLHQDWLNGKEYKCKVSNKALPAPIEKTISKAKGQPREPQVYTLPPSRDELTKNQVSLTCLVKGFYPSDIAVEWESNGQPENNYKTTPPVLDSDGSFFLYSKLTVDKSRWQQGNVFSCSVMHEALHNHYTQKSLSLSPGK

SEQ ID NO: 10 - protein, 232 aa, Mus musculus
PRGPTIKPCPPCKCPAPNLLGGPSVFIFPPKIKDVLMISLSPIVTCVVVDVSEDDPDVQISWFVNNVEVHTAQTQTHREDYNSTLRVVSALPIQHQDWMSGKEFKCKVNNKDLPAPIERTISKPKGSVRAPQVYVLPPPEEEMTKKQVTLTCMVTDFMPEDIYVEWTNNGKTELNYKNTEPVLDSDGSYFMYSKLRVEKKNWVERNSYSCSVVHEGLHNHHTTKSFSRTPGK

SEQ ID NO: 11 - protein, 330 aa, Homo sapiens
ASTKGPSVFPLAPSSKSTSGGTAALGCLVKDYFPEPVTVSWNSGALTSGVHTFPAVLQSSGLYSLSSVVTVPSSSLGTQTYICNVNHKPSNTKVDKRVEPKSCDKTHTCPPCPAPELLGGPSVFLFPPKPKDTLMISRTPEVTCVVVDVSHEDPEVKFNWYVDGVEVHNAKTKPREEQYNSTYRVVSVLTVLHQDWLNGKEYKCKVSNKALPAPIEKTISKAKGQPREPQVYTLPPSREEMTKNQVSLTCLVKGFYPSDIAVEWESNGQPENNYKTTPPVLDSDGSFFLYSKLTVDKSRWQQGNVFSCSVMHEALHNHYTQKSLSLSPGK

SEQ ID NO: 12 - protein, 326 aa, Homo sapiens
ASTKGPSVFPLAPCSRSTSESTAALGCLVKDYFPEPVTVSWNSGALTSGVHTFPAVLQSSGLYSLSSVVTVPSSNFGTQTYTCNVDHKPSNTKVDKTVERKCCVECPPCPAPPVAGPSVFLFPPKPKDTLMISRTPEVTCVVVDVSHEDPEVQFNWYVDGVEVHNAKTKPREEQFNSTFRVVSVLTVVHQDWLNGKEYKCKVSNKGLPAPIEKTISKTKGQPREPQVYTLPPSREEMTKNQVSLTCLVKGFYPSDIAVEWESNGQPENNYKTTPPMLDSDGSFFLYSKLTVDKSRWQQGNVFSCSVMHEALHNHYTQKSLSLSPGK

SEQ ID NO: 13 - protein, 327 aa, Homo sapiens
ASTKGPSVFPLAPCSRSTSESTAALGCLVKDYFPEPVTVSWNSGALTSGVHTFPAVLQSSGLYSLSSVVTVPSSSLGTKTYTCNVDHKPSNTKVDKRVESKYGPPCPPCPAPEFLGGPSVFLFPPKPKDTLMISRTPEVTCVVVDVSQEDPEVQFNWYVDGVEVHNAKTKPREEQFNSTYRVVSVLTVLHQDWLNGKEYKCKVSNKGLPSSIEKTISKAKGQPREPQVYTLPPSQEEMTKNQVSLTCLVKGFYPSDIAVEWESNGQPENNYKTTPPVLDSDGSFFLYSRLTVDKSRWQEGNVFSCSVMHEALHNHYTQKSLSLSLGK

SEQ ID NO: 14 - protein, 324 aa, Mus musculus
AKTTPPSVYPLAPGSAAQTNSMVTLGCLVKGYFPEPVTVTWNSGSLSSGVHTFPAVLESDLYTLSSSVTVPSSPRPSETVTCNVAHPASSTKVDKKIVPRDCGCKPCICTVPEVSSVFIFPPKPKDVLTITLTPKVTCVVVDISKDDPEVQFSWFVDDVEVHTAQTQPREEQFNSTFRSVSELPIMHQDWLNGKEFKCRVNSAAFPAPIEKTISKTKGRPKAPQVYTIPPPKEQMAKDKVSLTCMITDFFPEDITVEWQWNGQPAENYKNTQPIMNTNGSYFVYSKLNVQKSNWEAGNTFTCSVLHEGLHNHHTEKSLSHSPGK

SEQ ID NO: 15 - protein, 330 aa, Mus musculus
AKTTAPSVYPLAPVCGDTTGSSVTLGCLVKGYFPEPVTLTWNSGSLSSGVHTFPAVLQSDLYTLSSSVTVTSSTWPSQSITCNVAHPASSTKVDKKIEPRGPTIKPCPPCKCPAPNLLGGPSVFIFPPKIKDVLMISLSPIVTCVVVDVSEDDPDVQISWFVNNVEVHTAQTQTHREDYNSTLRVVSALPIQHQDWMSGKEFKCKVNNKDLPAPIERTISKPKGSVRAPQVYVLPPPEEEMTKKQVTLTCMVTDFMPEDIYVEWTNNGKTELNYKNTEPVLDSDGSYFMYSKLRVEKKNWVERNSYSCSVVHEGLHNHHTTKSFSRTPGK

SEQ ID NO: 16 - protein, 107 aa, Homo sapiens [sequence omitted]

SEQ ID NO: 17 - protein, 106 aa, Homo sapiens
GQPKAAPSVTLFPPSSEELQANKATLVCLISDFYPGAVTVAWKADSSPVKAGVETTTPSKQSNNKYAASSYLSLTPEQWKSHRSYSCQVTHEGSTVEKTVAPTECS

SEQ ID NO: 18 - protein, 107 aa, Mus musculus
RADAAPTVSIFPPSSEQLTSGGASVVCFLNNFYPKDINVKWKIDGSERQNGVLNSWTDQDSKDSTYSMSSTLTLTKDEYERHNSYTCEATHKTSTSPIVKSFNRNEC

SEQ ID NO: 19 - protein, 106 aa, Mus musculus
GQPKSSPSVTLFPPSSEELETNKATLVCTITDFYPGVVTVDWKVDGTPVTQGMETTQPSKQSNNKYMASSYLTLTARAWERHSSYSCQVTHEGHTVEKSLSRADCS

SEQ ID NO: 20 - protein, 121 aa, Artificial Sequence
  the heavy chain variable region of the humanized antibody H1A10+L3E8-M1
QVQLVQSGAEVKKPGASVKVSCKASGYAFSNYWMNWVRQAPGQGLEWMGQIFPGDSDTDYDQKFQGRVTMTRDTSTSTVYMELSSLRSEDTAVYYCARAGYYRGYYAMDYWGQGTTVTVSS

SEQ ID NO: 21 - protein, 108 aa, Artificial Sequence
  the light chain variable region L3E8-M1 of the humanized antibody H1A10+L3E8-M1
EIVMTQSPATLSVSPGERATLSCSVSSSISSSNLHWYQQKPGQAPRPWIYGTSNLASGIPARFSGSGSGTEFTLTISSLQSEDFAVYYCQQWSSYPLTFGQGTKLEIK

SEQ ID NO: 22 - protein, 122 aa, Artificial Sequence
  the heavy chain variable region of the anti-human TSLP control antibody Tezepelumab
QMQLVESGGGVVQPGRSLRLSCAASGFTFRTYGMHWVRQAPGKGLEWVAVIWYDGSNKHYADSVKGRFTITRDNSKNTLNLQMNSLRAEDTAVYYCARAPQWELVHEAFDIWGQGTMVTVSS

SEQ ID NO: 23 - protein, 108 aa, Artificial Sequence
  the light chain variable region of the anti-human TSLP control antibody Tezepelumab
SYVLTQPPSVSVAPGQTARITCGGNNLGSKSVHWYQQKPGQAPVLVVYDDSDRPSWIPERFSGSNSGNTATLTISRGEAGDEADYYCQVWDSSSDHVVFGGGTKLTVL

SEQ ID NO: 24 - protein, 116 aa, Artificial Sequence
  the humanized heavy chain mutant H3B10-M1
QVTLKESGPVLVKPTETLTLTCTVSGFSLSSYDISWIRQPPGKALEWLGVIWSEGGTSYSTSLKSRLTISKDTSKSQVVLTMTNMDPVDTATYYCARDSDDGYLNWGQGTLVTVSS

SEQ ID NO: 25 - protein, 108 aa, Artificial Sequence
  L3E8-M2
EIVMTQSPATLSVSPGERATLSCSVSSSISSSNLHWYQQKPGQAPKPWIYGTSNLASGIPARFSGSGSGTEFTLTISSLQSEDFAVYYCQQWSSYPLTFGQGTKLEIK

SEQ ID NO: 26 - protein, 108 aa, Artificial Sequence
  L3E8-M3
EIVMTQSPATLSVSPGERATITCSVSSSISSSNLHWYQQKPGQAPRPWIYGTSNLASGIPARFSGSGSGTEFTLTISSLQSEDFAVYYCQQWSSYPLTFGQGTKLEIK

SEQ ID NO: 27 - protein, 108 aa, Artificial Sequence
  L3E8-M4
EIVMTQSPATLSVSPGERATLSCSVSSSISSSNLHWYQQKPGQAPRPWIYGTSNLASGIPARFSGSGSGTEFTLTISSMEAEDFAVYYCQQWSSYPLTFGQGTKLEIK

SEQ ID NO: 28 - protein, 108 aa, Artificial Sequence
  the mutant L3E8-M7
EIVMTQSPATLSVSPGERATLSCSVSSSISSSNLHWYQQKPGQAPRPWIYGTSNLASGIPARFSGSGSGTEFTLTISSVQAEDFAVYYCQQWSSYPLTFGQGTKLEIK

SEQ ID NO: 29 - protein, 5 aa, Artificial Sequence
  HCDR1 of the humanized heavy chain mutant H3B10-M1
SYDIS

SEQ ID NO: 30 - protein, 16 aa, Artificial Sequence
  HCDR2 of the humanized heavy chain mutant H3B10-M1
VIWSEGGTSYSTSLKS

SEQ ID NO: 31 - protein, 8 aa, Artificial Sequence
  HCDR3 of the humanized heavy chain mutant H3B10-M1
DSDDGYLN

SEQ ID NO: 32 - protein, 12 aa, Artificial Sequence
  LCDR1 of the light chain variable region L3E8-M1
SVSSSISSSNLH

SEQ ID NO: 33 - protein, 7 aa, Artificial Sequence
  LCDR2 of the light chain variable region L3E8-M1
GTSNLAS

SEQ ID NO: 34 - protein, 9 aa, Artificial Sequence
  LCDR3 of the light chain variable region L3E8-M1
QQWSSYPLT

SEQ ID NO: 35 - protein, 5 aa, Artificial Sequence
  HCDR1 of the heavy chain variable region of the humanized antibody H1A10+L3E8-M1
NYWMN

SEQ ID NO: 36 - protein, 17 aa, Artificial Sequence
  HCDR2 of the heavy chain variable region of the humanized antibody H1A10+L3E8-M1
QIFPGDSDTDYDQKFQG

SEQ ID NO: 37 - protein, 12 aa, Artificial Sequence
  HCDR3 of the heavy chain variable region of the humanized antibody H1A10+L3E8-M1
AGYYRGYYAMDY

SEQ ID NO: 38 - protein, 446 aa, Artificial Sequence
  H3B10-M1-IgG1m3-H
QVTLKESGPVLVKPTETLTLTCTVSGFSLSSYDISWIRQPPGKALEWLGVIWSEGGTSYSTSLKSRLTISKDTSKSQVVLTMTNMDPVDTATYYCARDSDDGYLNWGQGTLVTVSSASTKGPSVFPLAPSSKSTSEGTAALGCLVKDYFPEPVTVSWNSGALTSGVHTFPAVLQSSGLYSLSSVVTVPSSSLGTQTYICNVDHKPSNTKVDKTVEPKSCDKTHTCPPCPAPEFEGGPSVFLFPPKPKDTLMISRTPEVTCVVVDVSQEDPEVQFNWYVDGVEVHNAKTKPREEQYNSTYRVVSVLTVLHQDWLNGKEYKCKVSNKALPASIEKTISKAKGQPREPQVCTLPPSQEEMTKNQVSLSCAVKGFYPSDIAVEWESNGQPENNYKTTPPVLDSDGSFFLVSKLTVDKSRWQEGNVFSCSVMHEALHNHYTQKSLSLSPGK

SEQ ID NO: 39 - protein, 215 aa, Artificial Sequence
  the light chain comprising the L3E8-M1 light chain variable region
EIVMTQSPATLSVSPGERATLSCSVSSSISSSNLHWYQQKPGQAPRPWIYGTSNLASGIPARFSGSGSGTEFTLTISSLQSEDFAVYYCQQWSSYPLTFGQGTKLEIKRTVAAPSVFIFPPSDEQLKSGTASVVCLLNNFYPREAKVQWKVDNALQSGNSQESVTEQDSKDSTYSLSSTLTLSKADYEKHKVYACEVTHQGLSSPVTKSFNRGEC

SEQ ID NO: 40 - protein, 215 aa, Artificial Sequence
  the light chain comprising the L3E8-M7 light chain variable region
EIVMTQSPATLSVSPGERATLSCSVSSSISSSNLHWYQQKPGQAPRPWIYGTSNLASGIPARFSGSGSGTEFTLTISSVQAEDFAVYYCQQWSSYPLTFGQGTKLEIKRTVAAPSVFIFPPSDEQLKSGTASVVCLLNNFYPREAKVQWKVDNALQSGNSQESVTEQDSKDSTYSLSSTLTLSKADYEKHKVYACEVTHQGLSSPVTKSFNRGEC

SEQ ID NO: 41 - protein, 451 aa, Artificial Sequence
  H1A10-IgG1m3-K
QVQLVQSGAEVKKPGASVKVSCKASGYAFSNYWMNWVRQAPGQGLEWMGQIFPGDSDTDYDQKFQGRVTMTRDTSTSTVYMELSSLRSEDTAVYYCARAGYYRGYYAMDYWGQGTTVTVSSASTKGPSVFPLAPSSKSTSGGTAALGCLVKDYFPEPVTVSWNSGALTSGVHTFPAVLQSSGLYSLSSVVTVPSSSLGTQTYICNVNHKPSNTKVDKRVEPKSCDKTHTCPPCPAPEFEGGPSVFLFPPKPKDTLMISRTPEVTCVVVDVSHEDPEVKFNWYVDGVEVHNAKTKPREEQYNSTYRVVSVLTVLHQDWLNGKEYKCKVSNKALPASIEKTISKAKGQPREPQVYTLPPCREEMTKNQVSLWCLVKGFYPSDIAVEWESNGQPENNYKTTPPVLDSDGSFFLYSKLTVDKSRWQQGNVFSCSVMHEALHNHYTQKSLSLSPGK

SEQ ID NO: 42 - protein, 209 aa, Homo sapiens
QGGAAEGVQIQIIYFNLETVQVTWNASKYSRTNLTFHYRFNGDEAYDQCTNYLLQEGHTSGCLLDAEQRDDILYFSIRNGTHPVFTASRWMVYYLKPSSPKHVRFSWHQDAVTVTCSDLSYGDLLYEVQYRSPFDTEWQSKQENTCNVTIEGLDAEKCYSFWVRVKAMEDVYGPDTYPSDWSEVTCWQRGEIRDACAETPTPPKPKLSK

SEQ ID NO: 43 - protein, 219 aa, Homo sapiens
ESGYAQNGDLEDAELDDYSFSCYSQLEVNGSQHSLTCAFEDPDVNTTNLEFEICGALVEVKCLNFRKLQEIYFIETKKFLLIGKSNICVKVGEKSLTCKKIDLTTIVKPEAPFDLSVIYREGANDFVVTFNTSHLQKKYVKVLMHDVAYRQEKDENKWTHVNLSSTKLTLLQRKLQPAAMYEIKVRSIPDHYFKGFWSEWSPSYYFRTPEINNSSGEMD